European Patent Specification EP 3 325 512 B1, published September 6, 2023. Title: MULTIVALENT AND MULTISPECIFIC GITR-BINDING FUSION PROTEINS. Applicant: INHIBRX LP Timmer, John C. Jones, Kyle S. Razai, Amir S. Hussain, Abrahim Willis, Katelyn M. Deveraux, Quinn Eckelman, Brendan P. The sequence listing filed with the application follows.

SEQUENCE LISTING (150 sequences)

SEQ ID NO: 1 - protein, 218 aa, Artificial Sequence
  chemically synthesized
PAPELLGGPSVFLFPPKPKDTLMISRTPEVTCVVVDVSHEDPEVKFNWYVDGVEVHNAKTKPREEQYNSTYRVVSVLTVLHQDWLNGKEYKCKVSNKALPAPIEKTISKAKGQPREPQVYTLPPSRDELTKNQVSLTCLVKGFYPSDIAVEWESNGQPENNYKTTPPVLDSDGSFFLYSKLTVDKSRWQQGNVFSCSVMHEALHNHYTQKSLSLSPGK

SEQ ID NO: 2 - protein, 215 aa, Artificial Sequence
  chemically synthesized
PAPGGPSVFLFPPKPKDTLMISRTPEVTCVVVDVSHEDPEVKFNWYVDGVEVHNAKTKPREEQYNSTYRVVSVLTVLHQDWLNGKEYKCKVSNKALPAPIEKTISKAKGQPREPQVYTLPPSRDELTKNQVSLTCLVKGFYPSDIAVEWESNGQPENNYKTTPPVLDSDGSFFLYSKLTVDKSRWQQGNVFSCSVMHEALHNHYTQKSLSLSPGK

SEQ ID NO: 3 - protein, 217 aa, Artificial Sequence
  chemically synthesized
PAPPVAGPSVFLFPPKPKDTLMISRTPEVTCVVVDVSHEDPEVQFNWYVDGVEVHNAKTKPREEQFNSTFRVVSVLTVVHQDWLNGKEYKCKVSNKGLPAPIEKTISKTKGQPREPQVYTLPPSREEMTKNQVSLTCLVKGFYPSDISVEWESNGQPENNYKTTPPMLDSDGSFFLYSKLTVDKSRWQQGNVFSCSVMHEALHNHYTQKSLSLSPGK

SEQ ID NO: 4 - protein, 218 aa, Artificial Sequence
  chemically synthesized
PAPELLGGPSVFLFPPKPKDTLMISRTPEVTCVVVDVSHEDPEVQFKWYVDGVEVHNAKTKPREEQYNSTFRVVSVLTVLHQDWLNGKEYKCKVSNKALPAPIEKTISKTKGQPREPQVYTLPPSREEMTKNQVSLTCLVKGFYPSDIAVEWESSGQPENNYNTTPPMLDSDGSFFLYSKLTVDKSRWQQGNIFSCSVMHEALHNRFTQKSLSLSPGK

SEQ ID NO: 5 - protein, 218 aa, Artificial Sequence
  chemically synthesized
PAPEFLGGPSVFLFPPKPKDTLMISRTPEVTCVVVDVSQEDPEVQFNWYVDGVEVHNAKTKPREEQFNSTYRVVSVLTVLHQDWLNGKEYKCKVSNKGLPSSIEKTISKAKGQPREPQVYTLPPSQEEMTKNQVSLTCLVKGFYPSDIAVEWESNGQPENNYKTTPPVLDSDGSFFLYSRLTVDKSRWQEGNVFSCSVMHEALHNHYTQKSLSLSLGK

SEQ ID NO: 6 - protein, 218 aa, Artificial Sequence
  chemically synthesized
PAPELLGGPSVFLFPPKPKDTLMISRTPEVTCVVVDVSQEDPEVQFNWYVDGVEVHNAKTKPREEQFNSTYRVVSVLTVLHQDWLNGKEYKCKVSNKGLPSSIEKTISKAKGQPREPQVYTLPPSQEEMTKNQVSLTCLVKGFYPSDIAVEWESNGQPENNYKTTPPVLDSDGSFFLYSRLTVDKSRWQEGNVFSCSVMHEALHNHYTQKSLSLSLGK

SEQ ID NO: 7 - protein, 14 aa, Artificial Sequence
  chemically synthesized
EPKSSDKTHTCPPC

SEQ ID NO: 8 - protein, 9 aa, Artificial Sequence
  chemically synthesized
DKTHTCPPC

SEQ ID NO: 9 - protein, 11 aa, Artificial Sequence
  chemically synthesized
ESKYGPPCPPC

SEQ ID NO: 10 - protein, 12 aa, Artificial Sequence
  chemically synthesized
GQGTLVTVKPGG

SEQ ID NO: 11 - protein, 12 aa, Artificial Sequence
  chemically synthesized
GQGTLVTVEPGG

SEQ ID NO: 12 - protein, 6 aa, Artificial Sequence
  chemically synthesized
GGSGGS

SEQ ID NO: 13 - protein, 9 aa, Artificial Sequence
  chemically synthesized
GGSGGSGGS

SEQ ID NO: 14 - protein, 12 aa, Artificial Sequence
  chemically synthesized
GGSGGSGGSGGS

SEQ ID NO: 15 - protein, 15 aa, Artificial Sequence
  chemically synthesized
GGSGGSGGSGGSGGS

SEQ ID NO: 16 - protein, 4 aa, Artificial Sequence
  chemically synthesized
GGGG

SEQ ID NO: 17 - protein, 5 aa, Artificial Sequence
  chemically synthesized
GGGGG

SEQ ID NO: 18 - protein, 6 aa, Artificial Sequence
  chemically synthesized
GGGGGG

SEQ ID NO: 19 - protein, 120 aa, Artificial Sequence
  chemically synthesized
  misc_feature (10)..(10): Xaa can be any naturally occurring amino acid
QVQLQESGGXLVQSGGSLRLSCAASGSVFSIDAMGWYRLAPGKQRELVAVMSSGSPKYADSVKGRFTISRGSARGTVYLQMDSLKPEDTAVYYCYADVATGWGRDASAYWGQGTQVTVSS

SEQ ID NO: 20 - protein, 121 aa, Artificial Sequence
  chemically synthesized
QVQLQQSGGGLVRAGGSLRLSCVAAGSTFSVNSMAWYRQAPGKERELVAAFTGGSTMNYASSVKGRFTISRGNAAHTVLLQMTNLKPEDTAVYYCNAEVNEGWNADYHDYWGQGTQVTVSS

SEQ ID NO: 21 - protein, 121 aa, Artificial Sequence
  chemically synthesized
QVQLVQSGGGLVQAGGSLRLSCTASGSIFSINHMAWYRQAPGKQREMVAHITGGASTKYADSVKGRFTISRDSALNTVSLRMNSLKPEDTAVYYCNAEVNEGWNADYYDVWGQGTQVTVSS

SEQ ID NO: 22 - protein, 121 aa, Artificial Sequence
  chemically synthesized
QVQLQESGGGLVQAGGSLRLSCAASGSVFSIDAMGWYRLAPGQQRELVAVLNGISSAKYADSVKGRFTISGDSAKNAVYLQMDGLKPEDTAVYYCYADVSTGWGRDAHGYWGQGTQVTVSS

SEQ ID NO: 23 - protein, 117 aa, Artificial Sequence
  chemically synthesized
EVQLVQSGGGLVQPGGSLRLSCAASGNIFSIDAMGWYRQAPGRQRELVAQIPGGPTDSVKGRFTVSGNSAKNTGYLQMNTLKPEDTAVYYCNIVASTSWGSPSKVYWGQGTQATVSS

SEQ ID NO: 24 - protein, 120 aa, Artificial Sequence
  chemically synthesized
QVQLQESGGGLVQPGGSLRLSCAASGSVFSIDSMSWFRQAPGNERELVALITGGRTTTYADSVKGRFTISRASAPNTVYLQMNSLKPEDTAVYYCNAVVSTGWGRNADDYWGQGTQVTVS

SEQ ID NO: 25 - protein, 119 aa, Artificial Sequence
  chemically synthesized
QVQLQQSGGGLVQAGGSLRLSCAASGSIFSIDAMGWYRLAPGKQRELVAVIDGVSPNYADSVKGRFTISSDIAKNTVYLQMHSPKPEDTAVYYCNADVSTGWGRPADHYWGQGTQVTVS

SEQ ID NO: 26 - protein, 120 aa, Artificial Sequence
  chemically synthesized
QVQLQESGGGLVQPGGSLRLSCAASGSVFSIDSMSWFRQAPGNERELVALITGGHTTTYGDSVKGRFTISRASAPNTVHLQMNSLQPEDTAVYYCNAAVSTGWGRNADDYWGQGTQVTVS

SEQ ID NO: 27 - protein, 118 aa, Artificial Sequence
  chemically synthesized
QLVQSGGGLVQPGESLRLSCAASGSVFSIDSVSWFRQGPGNERELVALITGGRTTTYADSVKGRFTISRANAPNTVHLRMNSLKPEDTAVYYCNAAVSTGWGRNADDYWGQGTQVTVS

SEQ ID NO: 28 - protein, 120 aa, Artificial Sequence
  chemically synthesized
QVQLVQSGGGLVQPGGSLRLICAASGSVFSIDSMSWFRQRPGNERELVALITGGRTTTYSDSVKGRFTISRASALNTVHLQMNSLKPEDTAVYYCNAALSTGWGRDASAYWGQGTQVTVS

SEQ ID NO: 29 - protein, 120 aa, Artificial Sequence
  chemically synthesized
QVQLQESGGGLVQAGGSLRLSCTASGSIFSINHMAWYRQAPGKQREMVAHITGGASTKYADSVKGRFTISRDSALNTVSLRMNSLKPEDTAVYYCNAEVNEGWNADYYDVWGQGTQVTVS

SEQ ID NO: 30 - protein, 119 aa, Artificial Sequence
  chemically synthesized
QLQLQESGGGTVQAGGSLRLSCAASRSIASINVMGWYRQAPGNQHELVAAITSGGSPNYAGSVRGRFIISRDNAKNTVYLQMNDLKPEDTAVYYCAGELRDDSNGYLHYWGQGTQVTVS

SEQ ID NO: 31 - protein, 120 aa, Artificial Sequence
  chemically synthesized
QVQLQESGGGLVQPGGSLRLSCAASGSVFSIDSMSWFRQTPGNERELVAHITGGRTTTYADSVKGRFTISRASAPNTVHLQMNNLKPEDTAVYYCNAAVSTGWGRNADDYWGQGTQVTVS

SEQ ID NO: 32 - protein, 119 aa, Artificial Sequence
  chemically synthesized
QVQLQESGGGLVQAGGSLRLSCTASGSIFSIDDMGWYRLAPGKQRELVAVHSGSSTNYGDSVKGRFTISGDSAKNTVYLQMHRLEPEDTAVYYCYAAISSGWGRDAEDYWGQGTQVTVS

SEQ ID NO: 33 - protein, 120 aa, Artificial Sequence
  chemically synthesized
QVQLVQSGGGLVQPGESLRLSCAASGSVFSIDSMSWFRQGPGNERELVALITGGRTTTYADSVKGRFTISRANAPNTVHLQMNSLKPEDTAVYYCNAAVSTGWGRSADDYWGQGTQVTVS

SEQ ID NO: 34 - protein, 120 aa, Artificial Sequence
  chemically synthesized
QVQLVQSGGGLVQPGESLRLSCAASGSVFSIDSMSWFRQGPGNERELVALITGGRTTTYADSVKGRFTISRANAPNTVHLQMNSLEPEDTAVYYCNAAVSTGWGRNADDYWGQGTQVTVS

SEQ ID NO: 35 - protein, 120 aa, Artificial Sequence
  chemically synthesized
QVQLVQSGGGLVQPGGSLRLSCAASGSVFSIDSMSWFRQAPGNERELVALITGGRTTTYADSVKGRFTISRASAPNTVHLQMNSLKPEDTAVYYCNAVVSTGWGRNADDYWGQGTQVTVS

SEQ ID NO: 36 - protein, 121 aa, Artificial Sequence
  chemically synthesized
EVQLLESGGGEVQPGGSLRLSCAASGSVFSIDAMSWFRQAPGKGLELVSAITGGRTTYYAESVKGRFTISRDNAKNTLYLQMSSLRAEDTAVYYCNAVVSTGWGRNADDYWGQGTLVTVKP

SEQ ID NO: 37 - protein, 121 aa, Artificial Sequence
  chemically synthesized
EVQLLESGGGEVQPGGSLRLSCAASGSVFSIDAMSWFRQAPGKGLELVCAITGGRTTYYAESVKGRFTCSRDNAKNTLYLQMSSLRAEDTAVYYCNAVVSTGWGRNADDYWGQGTLVTVKP

SEQ ID NO: 38 - protein, 121 aa, Artificial Sequence
  chemically synthesized
EVQLLESGGGEVQPGGSLRLSCAASGSVFSIDSMSWFRQAPGKGLELVSLITGGRTTYYAESVKGRFTISRDNAKNTLYLQMSSLRAEDTAVYYCNAVVSTGWGRNADDYWGQGTLVTVKP

SEQ ID NO: 39 - protein, 121 aa, Artificial Sequence
  chemically synthesized
EVQLLESGGGEVQPGGSLRLSCAASGSVFSIDSMSWFRQAPGKGLELVCLITGGRTTYYAESVKGRFTCSRDNAKNTLYLQMSSLRAEDTAVYYCNAVVSTGWGRNADDYWGQGTLVTVKP

SEQ ID NO: 40 - protein, 121 aa, Artificial Sequence
  chemically synthesized
EVQLLESGGGEVQPGGSLRLSCAASGSVFSIDAMSWFRQAPGKGLELVSLITGGRTTYYAESVKGRFTISRDNAKNTLYLQMSSLRAEDTAVYYCNAVVSTGWGRNADDYWGQGTLVTVKP

SEQ ID NO: 41 - protein, 121 aa, Artificial Sequence
  chemically synthesized
EVQLLESGGGEVQPGGSLRLSCAASGSVFSIDAMSWFRQAPGKGLELVCLITGGRTTYYAESVKGRFTCSRDNAKNTLYLQMSSLRAEDTAVYYCNAVVSTGWGRNADDYWGQGTLVTVKP

SEQ ID NO: 42 - protein, 119 aa, Artificial Sequence
  chemically synthesized
EVQLLESGGGEVQPGGSLRLSCAASGSVFSIDAMGWYRQAPGKGLELVSALSGISSATYAESVKGRFTISRDNAKNTLYLQMSSLRAEDTAVYYCYADVSTGWGRDAHGYWGQGTLVTV

SEQ ID NO: 43 - protein, 119 aa, Artificial Sequence
  chemically synthesized
EVQLLESGGGEVQPGGSLRLSCAASGSVFSIDAMGWYRQAPGKGRELVSALSGISSATYAESVKGRFTISRDNAKNTLYLQMSSLRAEDTAVYYCYADVSTGWGRDAHGYWGQGTLVTV

SEQ ID NO: 44 - protein, 119 aa, Artificial Sequence
  chemically synthesized
EVQLLESGGGEVQPGGSLRLSCAASGSVFSIDAMGWYRQAPGKQRELVSALSGISSATYAESVKGRFTISRDNAKNTLYLQMSSLRAEDTAVYYCYADVSTGWGRDAHGYWGQGTLVTV

SEQ ID NO: 45 - protein, 119 aa, Artificial Sequence
  chemically synthesized
EVQLLESGGGEVQPGGSLRLSCAASGSVFSIDAMGWYRQAPGQQRELVSALSGISSATYAESVKGRFTISRDNAKNTLYLQMSSLRAEDTAVYYCYADVSTGWGRDAHGYWGQGTLVTV

SEQ ID NO: 46 - protein, 119 aa, Artificial Sequence
  chemically synthesized
EVQLLESGGGEVQPGGSLRLSCAASGSVFSIDAMGWYRQAPGKGLELVAVLSGISSATYAESVKGRFTISRDNAKNTLYLQMSSLRAEDTAVYYCYADVSTGWGRDAHGYWGQGTLVTV

SEQ ID NO: 47 - protein, 119 aa, Artificial Sequence
  chemically synthesized
EVQLLESGGGEVQPGGSLRLSCAASGSVFSIDAMGWYRQAPGKGRELVAVLSGISSATYAESVKGRFTISRDNAKNTLYLQMSSLRAEDTAVYYCYADVSTGWGRDAHGYWGQGTLVTV

SEQ ID NO: 48 - protein, 119 aa, Artificial Sequence
  chemically synthesized
EVQLLESGGGEVQPGGSLRLSCAASGSVFSIDAMGWYRQAPGKQRELVAVLSGISSATYAESVKGRFTISRDNAKNTLYLQMSSLRAEDTAVYYCYADVSTGWGRDAHGYWGQGTLVTV

SEQ ID NO: 49 - protein, 119 aa, Artificial Sequence
  chemically synthesized
EVQLLESGGGEVQPGGSLRLSCAASGSVFSIDAMGWYRQAPGQQRELVAVLSGISSATYAESVKGRFTISRDNAKNTLYLQMSSLRAEDTAVYYCYADVSTGWGRDAHGYWGQGTLVTV

SEQ ID NO: 50 - protein, 119 aa, Artificial Sequence
  chemically synthesized
EVQLLESGGGEVQPGGSLRLSCAASGSVFSIDAMGWYRQAPGKQRELVAVLSGISSAKYAESVKGRFTISRDNAKNTLYLQMSSLRAEDTAVYYCYADVSTGWGRDAHGYWGQGTLVTV

SEQ ID NO: 51 - protein, 119 aa, Artificial Sequence
  chemically synthesized
EVQLLESGGGEVQPGGSLRLSCAASGSVFSIDAMGWYRLAPGQQRELVAVLSGISSAKYAESVKGRFTISRDNAKNTLYLQMSSLRAEDTAVYYCYADVSTGWGRDAHGYWGQGTLVTV

SEQ ID NO: 52 - protein, 119 aa, Artificial Sequence
  chemically synthesized
EVQLLESGGGEVQPGGSLRLSCAASGSVFSIDAMGWYRQAPGKQRELVAVLSGISSAKYADSVKGRFTISGDNAKNTLYLQMSSLRAEDTAVYYCYADVSTGWGRDAHGYWGQGTLVTV

SEQ ID NO: 53 - protein, 119 aa, Artificial Sequence
  chemically synthesized
EVQLLESGGGEVQPGGSLRLSCAASGSVFSIDAMGWYRQAPGKQRELVAVLSGISSAKYAESVKGRFTISRDSAKNAVYLQMDGLKPEDTAVYYCYADVSTGWGRDAHGYWGQGTLVTV

SEQ ID NO: 54 - protein, 119 aa, Artificial Sequence
  chemically synthesized
EVQLLESGGGEVQPGGSLRLSCAASGSVFSIDAMGWYRQAPGKQRELVAVLSGISSAKYAESVKGRFTISRDNAKNTVYLQMSSLRAEDTAVYYCYADVSTGWGRDAHGYWGQGTLVTV

SEQ ID NO: 55 - protein, 119 aa, Artificial Sequence
  chemically synthesized
EVQLLESGGGEVQPGGSLRLSCAASGSVFSIDAMGWYRQAPGKQRELVAVLSGISSAKYAESVKGRFTISRASAPNTLYLQMSSLRAEDTAVYYCYADVSTGWGRDAHGYWGQGTLVTV

SEQ ID NO: 56 - protein, 119 aa, Artificial Sequence
  chemically synthesized
EVQLLESGGGEVQPGGSLRLSCAASGSVFSIDAMGWYRQAPGKQRELVAVLSGISSAKYAESVKGRFTISRASAPNTVYLQMSSLRAEDTAVYYCYADVSTGWGRDAHGYWGQGTLVTV

SEQ ID NO: 57 - protein, 119 aa, Artificial Sequence
  chemically synthesized
EVQLLESGGGEVQPGGSLRLSCAASGSVFSIDAMGWYRQAPGKQRELVAVLSGISSAKYAASAPGRFTISRDAVKNTVYLQMSSLRAEDTAVYYCYADVSTGWGRDAHGYWGQGTLVTV

SEQ ID NO: 58 - protein, 119 aa, Artificial Sequence
  chemically synthesized
EVQLLESGGGEVQPGGSLRLSCAASGSVFSIDAMGWYRQAPGKQRELVAVLSGISSAKYAASAPGRFTISRDAVENTVYLQMSSLRAEDTAVYYCYADVSTGWGRDAHGYWGQGTLVTV

SEQ ID NO: 59 - protein, 119 aa, Artificial Sequence
  chemically synthesized
EVQLLESGGGEVQPGGSLRLSCAASGSVFSIDAMGWYRQAPGKQRELVAVLSGISSAKYAASAPGRFTISRDNAKNTVYLQMSSLRAEDTAVYYCYADVSTGWGRDAHGYWGQGTLVTV

SEQ ID NO: 60 - protein, 119 aa, Artificial Sequence
  chemically synthesized
EVQLLESGGGEVQPGGSLRLSCAASGSVFSIDAMGWYRQAPGKQRELVAVLSGISSAKYADAVKGRFTISRASAPNTVYLQMSSLRAEDTAVYYCYADVSTGWGRDAHGYWGQGTLVTV

SEQ ID NO: 61 - protein, 119 aa, Artificial Sequence
  chemically synthesized
EVQLLESGGGEVQPGGSLRLSCAASGSVFSIDAMGWYRQAPGKQRELVAVLSGISSAKYADAVEGRFTISRASAPNTVYLQMSSLRAEDTAVYYCYADVSTGWGRDAHGYWGQGTLVTV

SEQ ID NO: 62 - protein, 119 aa, Artificial Sequence
  chemically synthesized
EVQLLESGGGEVQPGGSLRLSCAASGSVFSIDAMGWYRQAPGKQRELVAVLSGISSAKYAASAPGRFTISRASAPNTVYLQMSSLRAEDTAVYYCYADVSTGWGRDAHGYWGQGTLVTV

SEQ ID NO: 63 - protein, 110 aa, Artificial Sequence
  chemically synthesized
EVQLLESGGGEVQPGGSLRLSCAASGFTFSTHGMDWFRQAPGKDLEWVSAINNGGSWTSYASSVKGRFTISRDNAKNTLYLQMSSLRAEDTAVYWCQNRVTRGQGTLVTV

SEQ ID NO: 64 - protein, 110 aa, Artificial Sequence
  chemically synthesized
EVQLLESGGGEVQPGGSLRLSCAASGFTFSTHGMDWFRQAPGKDLEWVSAINNGGSWTSYASSVKGRFTISRDNAKNTLYLQMSSLRAEDTAVYYCQNRVTRGQGTLVTV

SEQ ID NO: 65 - protein, 110 aa, Artificial Sequence
  chemically synthesized
EVQLLESGGGEVQPGGSLRLSCAASGFTFSTHGMDWFRQAPGKDLEWVSAINQGGSWTSYASSVKGRFTISRDNAKNTLYLQMSSLRAEDTAVYYCQNRVTRGQGTLVTV

SEQ ID NO: 66 - protein, 110 aa, Artificial Sequence
  chemically synthesized
EVQLLESGGGEVQPGGSLRLSCAASGFTFSTHGMDWFRQAPGKGLEWVSAINNGGSWTSYASSVKGRFTISRDNAKNTLYLQMSSLRAEDTAVYWCQNRVTRGQGTLVTV

SEQ ID NO: 67 - protein, 110 aa, Artificial Sequence
  chemically synthesized
EVQLLESGGGEVQPGGSLRLSCAASGFTFSTHGMDWFRQAPGKGLEWVSAINNGGSWTSYASSVKGRFTISRDNAKNTLYLQMSSLRAEDTAVYYCQNRVTRGQGTLVTV

SEQ ID NO: 68 - protein, 110 aa, Artificial Sequence
  chemically synthesized
EVQLLESGGGEVQPGGSLRLSCAASGFTFSTHGMDWFRQAPGKDLEWVSAIQSGGSWTSYASSVKGRFTISRDNAKNTLYLQMSSLRAEDTAVYWCQNRVTRGQGTLVTV

SEQ ID NO: 69 - protein, 110 aa, Artificial Sequence
  chemically synthesized
EVQLLESGGGEVQPGGSLRLSCAASGFTFSTHGMDWFRQAPGKDLEWVSAIQSGGSWTSYASSVKGRFTISRDNAKNTLYLEMNNLKPEDTAVYWCQNRVTRGQGTLVTV

SEQ ID NO: 70 - protein, 110 aa, Artificial Sequence
  chemically synthesized
EVQLLESGGGEVQPGGSLRLSCAASGFTFSTHGMDWFRQAPGKDLEWVSAIQSGGSWTSYASSVKGRFTISRDNAKNTLYLQMNNLRAEDTAVYWCQNRVTRGQGTLVTV

SEQ ID NO: 71 - protein, 110 aa, Artificial Sequence
  chemically synthesized
EVQLLESGGGEVQPGGSLRLSCAASGFTFSTHGMDWFRQAPGKDLEWVSAIQSGGSWTSYASSVKGRFTISRDNAKNTLYLEMSSLRAEDTAVYWCQNRVTRGQGTLVTV

SEQ ID NO: 72 - protein, 110 aa, Artificial Sequence
  chemically synthesized
EVQLLESGGGEVQPGGSLRLSCAASGFTFSTHGMDWFRQAPGKDLEWVSAIQSGGSWTSYASSVKGRFTISRDNAKNTLYLQMSSLRPEDTAVYWCQNRVTRGQGTLVTV

SEQ ID NO: 73 - protein, 110 aa, Artificial Sequence
  chemically synthesized
EVQLLESGGGEVQPGGSLRLSCAASGFTFSTHGMDWFRQAPGKDLEWVSAIQSGGSWTSYASSVKGRFTISRDNAKNTLYLQMQQLRAEDTAVYWCQNRVTRGQGTLVTV

SEQ ID NO: 74 - protein, 110 aa, Artificial Sequence
  chemically synthesized
EVQLLESGGGEVQPGGSLRLSCAASGFTFSTHGMDWFRQAPGKDLEWVSAIQSGGSWTSYASSVKGRFTISRDNAKNTLYLQMQNLRAEDTAVYWCQNRVTRGQGTLVTV

SEQ ID NO: 75 - protein, 110 aa, Artificial Sequence
  chemically synthesized
EVQLLESGGGEVQPGGSLRLSCAASGFTFSTHGMDWFRQAPGKDLEWVSAIQSGGSWTSYASSVKGRFTISRDNAKNTLYLQMDNLRAEDTAVYWCQNRVTRGQGTLVTV

SEQ ID NO: 76 - protein, 110 aa, Artificial Sequence
  chemically synthesized
EVQLLESGGGEVQPGGSLRLSCAASGFTFSTHGMDWFRQAPGKDLEWVSAIQSGGSWTSYASSVKGRFTISRDNAKNTLYLQMNDLRAEDTAVYWCQNRVTRGQGTLVTV

SEQ ID NO: 77 - protein, 110 aa, Artificial Sequence
  chemically synthesized
EVQLLESGGGEVQPGGSLRLSCAASGFTFSTHGMDWFRQAPGKDLEWVSAIQSGGSWTSYASSVKGRFTISRDNAKNTLYLQMDDLRAEDTAVYWCQNRVTRGQGTLVTV

SEQ ID NO: 78 - protein, 110 aa, Artificial Sequence
  chemically synthesized
EVQLLESGGGEVQPGGSLRLSCAASGFTFSTHGMDWFRQAPGKDLEWVSAIQSGGSWTSYASSVKGRFTISRDNAKNTLYLQMQDLRAEDTAVYWCQNRVTRGQGTLVTV

SEQ ID NO: 79 - protein, 110 aa, Artificial Sequence
  chemically synthesized
EVQLLESGGGEVQPGGSLRLSCAASGFTFSTHGMDWFRQAPGKDLEWVSAIQSGGSWTSYASSVKGRFTISRDNAKNTLYLQMNQLRAEDTAVYWCQNRVTRGQGTLVTV

SEQ ID NO: 80 - protein, 110 aa, Artificial Sequence
  chemically synthesized
EVQLLESGGGEVQPGGSLRLSCAASGFTFSTHGMDWFRQAPGKDLEWVSAIQSGGSWTSYASSVKGRFTISRDNAKNTLYLQMSNLRAEDTAVYWCQNRVTRGQGTLVTV

SEQ ID NO: 81 - protein, 494 aa, Artificial Sequence
  chemically synthesized
MKWVTFISLLFLFSSAYSEVQLLESGGGEVQPGGSLRLSCAASGSVFSIDAMSWFRQAPGKGLELVSAITGGRTTYYAESVKGRFTISRDNAKNTLYLQMSSLRAEDTAVYYCNAVVSTGWGRNADDYWGQGTLVTVKPGGSGGSEVQLLESGGGEVQPGGSLRLSCAASGSVFSIDAMSWFRQAPGKGLELVSAITGGRTTYYAESVKGRFTISRDNAKNTLYLQMSSLRAEDTAVYYCNAVVSTGWGRNADDYWGQGTLVTVKPGGGGDKTHTCPPCPAPGGPSVFLFPPKPKDTLMISRTPEVTCVVVDVSHEDPEVKFNWYVDGVEVHNAKTKPREEQYNSTYRVVSVLTVLHQDWLNGKEYKCKVSNKALPAPIEKTISKAKGQPREPQVYTLPPSRDELTKNQVSLTCLVKGFYPSDIAVEWESNGQPENNYKTTPPVLDSDGSFFLYSKLTVDKSRWQQGNVFSCSVMHEALHNHYTQKSLSLSPGK

SEQ ID NO: 82 - protein, 494 aa, Artificial Sequence
  chemically synthesized
MKWVTFISLLFLFSSAYSEVQLLESGGGEVQPGGSLRLSCAASGSVFSIDAMSWFRQAPGKGLELVCAITGGRTTYYAESVKGRFTCSRDNAKNTLYLQMSSLRAEDTAVYYCNAVVSTGWGRNADDYWGQGTLVTVKPGGSGGSEVQLLESGGGEVQPGGSLRLSCAASGSVFSIDAMSWFRQAPGKGLELVCAITGGRTTYYAESVKGRFTCSRDNAKNTLYLQMSSLRAEDTAVYYCNAVVSTGWGRNADDYWGQGTLVTVKPGGGGDKTHTCPPCPAPGGPSVFLFPPKPKDTLMISRTPEVTCVVVDVSHEDPEVKFNWYVDGVEVHNAKTKPREEQYNSTYRVVSVLTVLHQDWLNGKEYKCKVSNKALPAPIEKTISKAKGQPREPQVYTLPPSRDELTKNQVSLTCLVKGFYPSDIAVEWESNGQPENNYKTTPPVLDSDGSFFLYSKLTVDKSRWQQGNVFSCSVMHEALHNHYTQKSLSLSPGK

SEQ ID NO: 83 - protein, 497 aa, Artificial Sequence
  chemically synthesized
MKWVTFISLLFLFSSAYSEVQLLESGGGEVQPGGSLRLSCAASGSVFSIDAMSWFRQAPGKGLELVSAITGGRTTYYAESVKGRFTISRDNAKNTLYLQMSSLRAEDTAVYYCNAVVSTGWGRNADDYWGQGTLVTVKPGGSGGSEVQLLESGGGEVQPGGSLRLSCAASGSVFSIDAMSWFRQAPGKGLELVSAITGGRTTYYAESVKGRFTISRDNAKNTLYLQMSSLRAEDTAVYYCNAVVSTGWGRNADDYWGQGTLVTVKPGGGGDKTHTCPPCPAPELLGGPSVFLFPPKPKDTLMISRTPEVTCVVVDVSHEDPEVKFNWYVDGVEVHNAKTKPREEQYNSTYRVVSVLTVLHQDWLNGKEYKCKVSNKALPAPIEKTISKAKGQPREPQVYTLPPSRDELTKNQVSLTCLVKGFYPSDIAVEWESNGQPENNYKTTPPVLDSDGSFFLYSKLTVDKSRWQQGNVFSCSVMHEALHNHYTQKSLSLSPGK

SEQ ID NO: 84 - protein, 497 aa, Artificial Sequence
  chemically synthesized
MKWVTFISLLFLFSSAYSEVQLLESGGGEVQPGGSLRLSCAASGSVFSIDAMSWFRQAPGKGLELVCAITGGRTTYYAESVKGRFTCSRDNAKNTLYLQMSSLRAEDTAVYYCNAVVSTGWGRNADDYWGQGTLVTVKPGGSGGSEVQLLESGGGEVQPGGSLRLSCAASGSVFSIDAMSWFRQAPGKGLELVCAITGGRTTYYAESVKGRFTCSRDNAKNTLYLQMSSLRAEDTAVYYCNAVVSTGWGRNADDYWGQGTLVTVKPGGGGDKTHTCPPCPAPELLGGPSVFLFPPKPKDTLMISRTPEVTCVVVDVSHEDPEVKFNWYVDGVEVHNAKTKPREEQYNSTYRVVSVLTVLHQDWLNGKEYKCKVSNKALPAPIEKTISKAKGQPREPQVYTLPPSRDELTKNQVSLTCLVKGFYPSDIAVEWESNGQPENNYKTTPPVLDSDGSFFLYSKLTVDKSRWQQGNVFSCSVMHEALHNHYTQKSLSLSPGK

SEQ ID NO: 85 - protein, 494 aa, Artificial Sequence
  chemically synthesized
MKWVTFISLLFLFSSAYSEVQLLESGGGEVQPGGSLRLSCAASGSVFSIDSMSWFRQAPGKGLELVSLITGGRTTYYAESVKGRFTISRDNAKNTLYLQMSSLRAEDTAVYYCNAVVSTGWGRNADDYWGQGTLVTVKPGGSGGSEVQLLESGGGEVQPGGSLRLSCAASGSVFSIDSMSWFRQAPGKGLELVSLITGGRTTYYAESVKGRFTISRDNAKNTLYLQMSSLRAEDTAVYYCNAVVSTGWGRNADDYWGQGTLVTVKPGGGGDKTHTCPPCPAPGGPSVFLFPPKPKDTLMISRTPEVTCVVVDVSHEDPEVKFNWYVDGVEVHNAKTKPREEQYNSTYRVVSVLTVLHQDWLNGKEYKCKVSNKALPAPIEKTISKAKGQPREPQVYTLPPSRDELTKNQVSLTCLVKGFYPSDIAVEWESNGQPENNYKTTPPVLDSDGSFFLYSKLTVDKSRWQQGNVFSCSVMHEALHNHYTQKSLSLSPGK

SEQ ID NO: 86 - protein, 494 aa, Artificial Sequence
  chemically synthesized
MKWVTFISLLFLFSSAYSEVQLLESGGGEVQPGGSLRLSCAASGSVFSIDSMSWFRQAPGKGLELVCLITGGRTTYYAESVKGRFTCSRDNAKNTLYLQMSSLRAEDTAVYYCNAVVSTGWGRNADDYWGQGTLVTVKPGGSGGSEVQLLESGGGEVQPGGSLRLSCAASGSVFSIDSMSWFRQAPGKGLELVCLITGGRTTYYAESVKGRFTCSRDNAKNTLYLQMSSLRAEDTAVYYCNAVVSTGWGRNADDYWGQGTLVTVKPGGGGDKTHTCPPCPAPGGPSVFLFPPKPKDTLMISRTPEVTCVVVDVSHEDPEVKFNWYVDGVEVHNAKTKPREEQYNSTYRVVSVLTVLHQDWLNGKEYKCKVSNKALPAPIEKTISKAKGQPREPQVYTLPPSRDELTKNQVSLTCLVKGFYPSDIAVEWESNGQPENNYKTTPPVLDSDGSFFLYSKLTVDKSRWQQGNVFSCSVMHEALHNHYTQKSLSLSPGK

SEQ ID NO: 87 - protein, 497 aa, Artificial Sequence
  chemically synthesized
MKWVTFISLLFLFSSAYSEVQLLESGGGEVQPGGSLRLSCAASGSVFSIDSMSWFRQAPGKGLELVSLITGGRTTYYAESVKGRFTISRDNAKNTLYLQMSSLRAEDTAVYYCNAVVSTGWGRNADDYWGQGTLVTVKPGGSGGSEVQLLESGGGEVQPGGSLRLSCAASGSVFSIDSMSWFRQAPGKGLELVSLITGGRTTYYAESVKGRFTISRDNAKNTLYLQMSSLRAEDTAVYYCNAVVSTGWGRNADDYWGQGTLVTVKPGGGGDKTHTCPPCPAPELLGGPSVFLFPPKPKDTLMISRTPEVTCVVVDVSHEDPEVKFNWYVDGVEVHNAKTKPREEQYNSTYRVVSVLTVLHQDWLNGKEYKCKVSNKALPAPIEKTISKAKGQPREPQVYTLPPSRDELTKNQVSLTCLVKGFYPSDIAVEWESNGQPENNYKTTPPVLDSDGSFFLYSKLTVDKSRWQQGNVFSCSVMHEALHNHYTQKSLSLSPGK

SEQ ID NO: 88 - protein, 497 aa, Artificial Sequence
  chemically synthesized
MKWVTFISLLFLFSSAYSEVQLLESGGGEVQPGGSLRLSCAASGSVFSIDSMSWFRQAPGKGLELVCLITGGRTTYYAESVKGRFTCSRDNAKNTLYLQMSSLRAEDTAVYYCNAVVSTGWGRNADDYWGQGTLVTVKPGGSGGSEVQLLESGGGEVQPGGSLRLSCAASGSVFSIDSMSWFRQAPGKGLELVCLITGGRTTYYAESVKGRFTCSRDNAKNTLYLQMSSLRAEDTAVYYCNAVVSTGWGRNADDYWGQGTLVTVKPGGGGDKTHTCPPCPAPELLGGPSVFLFPPKPKDTLMISRTPEVTCVVVDVSHEDPEVKFNWYVDGVEVHNAKTKPREEQYNSTYRVVSVLTVLHQDWLNGKEYKCKVSNKALPAPIEKTISKAKGQPREPQVYTLPPSRDELTKNQVSLTCLVKGFYPSDIAVEWESNGQPENNYKTTPPVLDSDGSFFLYSKLTVDKSRWQQGNVFSCSVMHEALHNHYTQKSLSLSPGK

SEQ ID NO: 89 - protein, 494 aa, Artificial Sequence
  chemically synthesized
MKWVTFISLLFLFSSAYSEVQLLESGGGEVQPGGSLRLSCAASGSVFSIDAMSWFRQAPGKGLELVSLITGGRTTYYAESVKGRFTISRDNAKNTLYLQMSSLRAEDTAVYYCNAVVSTGWGRNADDYWGQGTLVTVKPGGSGGSEVQLLESGGGEVQPGGSLRLSCAASGSVFSIDAMSWFRQAPGKGLELVSLITGGRTTYYAESVKGRFTISRDNAKNTLYLQMSSLRAEDTAVYYCNAVVSTGWGRNADDYWGQGTLVTVKPGGGGDKTHTCPPCPAPGGPSVFLFPPKPKDTLMISRTPEVTCVVVDVSHEDPEVKFNWYVDGVEVHNAKTKPREEQYNSTYRVVSVLTVLHQDWLNGKEYKCKVSNKALPAPIEKTISKAKGQPREPQVYTLPPSRDELTKNQVSLTCLVKGFYPSDIAVEWESNGQPENNYKTTPPVLDSDGSFFLYSKLTVDKSRWQQGNVFSCSVMHEALHNHYTQKSLSLSPGK

SEQ ID NO: 90 - protein, 494 aa, Artificial Sequence
  chemically synthesized
MKWVTFISLLFLFSSAYSEVQLLESGGGEVQPGGSLRLSCAASGSVFSIDAMSWFRQAPGKGLELVCLITGGRTTYYAESVKGRFTCSRDNAKNTLYLQMSSLRAEDTAVYYCNAVVSTGWGRNADDYWGQGTLVTVKPGGSGGSEVQLLESGGGEVQPGGSLRLSCAASGSVFSIDAMSWFRQAPGKGLELVCLITGGRTTYYAESVKGRFTCSRDNAKNTLYLQMSSLRAEDTAVYYCNAVVSTGWGRNADDYWGQGTLVTVKPGGGGDKTHTCPPCPAPGGPSVFLFPPKPKDTLMISRTPEVTCVVVDVSHEDPEVKFNWYVDGVEVHNAKTKPREEQYNSTYRVVSVLTVLHQDWLNGKEYKCKVSNKALPAPIEKTISKAKGQPREPQVYTLPPSRDELTKNQVSLTCLVKGFYPSDIAVEWESNGQPENNYKTTPPVLDSDGSFFLYSKLTVDKSRWQQGNVFSCSVMHEALHNHYTQKSLSLSPGK

SEQ ID NO: 91 - protein, 497 aa, Artificial Sequence
  chemically synthesized
MKWVTFISLLFLFSSAYSEVQLLESGGGEVQPGGSLRLSCAASGSVFSIDAMSWFRQAPGKGLELVSLITGGRTTYYAESVKGRFTISRDNAKNTLYLQMSSLRAEDTAVYYCNAVVSTGWGRNADDYWGQGTLVTVKPGGSGGSEVQLLESGGGEVQPGGSLRLSCAASGSVFSIDAMSWFRQAPGKGLELVSLITGGRTTYYAESVKGRFTISRDNAKNTLYLQMSSLRAEDTAVYYCNAVVSTGWGRNADDYWGQGTLVTVKPGGGGDKTHTCPPCPAPELLGGPSVFLFPPKPKDTLMISRTPEVTCVVVDVSHEDPEVKFNWYVDGVEVHNAKTKPREEQYNSTYRVVSVLTVLHQDWLNGKEYKCKVSNKALPAPIEKTISKAKGQPREPQVYTLPPSRDELTKNQVSLTCLVKGFYPSDIAVEWESNGQPENNYKTTPPVLDSDGSFFLYSKLTVDKSRWQQGNVFSCSVMHEALHNHYTQKSLSLSPGK

SEQ ID NO: 92 - protein, 497 aa, Artificial Sequence
  chemically synthesized
MKWVTFISLLFLFSSAYSEVQLLESGGGEVQPGGSLRLSCAASGSVFSIDAMSWFRQAPGKGLELVCLITGGRTTYYAESVKGRFTCSRDNAKNTLYLQMSSLRAEDTAVYYCNAVVSTGWGRNADDYWGQGTLVTVKPGGSGGSEVQLLESGGGEVQPGGSLRLSCAASGSVFSIDAMSWFRQAPGKGLELVCLITGGRTTYYAESVKGRFTCSRDNAKNTLYLQMSSLRAEDTAVYYCNAVVSTGWGRNADDYWGQGTLVTVKPGGGGDKTHTCPPCPAPELLGGPSVFLFPPKPKDTLMISRTPEVTCVVVDVSHEDPEVKFNWYVDGVEVHNAKTKPREEQYNSTYRVVSVLTVLHQDWLNGKEYKCKVSNKALPAPIEKTISKAKGQPREPQVYTLPPSRDELTKNQVSLTCLVKGFYPSDIAVEWESNGQPENNYKTTPPVLDSDGSFFLYSKLTVDKSRWQQGNVFSCSVMHEALHNHYTQKSLSLSPGK

SEQ ID NO: 93 - protein, 479 aa, Artificial Sequence
  chemically synthesized
EVQLLESGGGEVQPGGSLRLSCAASGSVFSIDAMGWYRQAPGKQRELVAVLSGISSAKYAASAPGRFTISRDNAKNTVYLQMSSLRAEDTAVYYCYADVSTGWGRDAHGYWGQGTLVTVKPGGSGGSEVQLLESGGGEVQPGGSLRLSCAASGSVFSIDAMGWYRQAPGKQRELVAVLSGISSAKYAASAPGRFTISRDNAKNTVYLQMSSLRAEDTAVYYCYADVSTGWGRDAHGYWGQGTLVTVKPGGGGDKTHTCPPCPAPELLGGPSVFLFPPKPKDTLMISRTPEVTCVVVDVSHEDPEVKFNWYVDGVEVHNAKTKPREEQYNSTYRVVSVLTVLHQDWLNGKEYKCKVSNKALPAPIEKTISKAKGQPREPQVYTLPPSRDELTKNQVSLTCLVKGFYPSDIAVEWESNGQPENNYKTTPPVLDSDGSFFLYSKLTVDKSRWQQGNVFSCSVMHEALHNHYTQKSLSLSPGK

SEQ ID NO: 94 - protein, 621 aa, Artificial Sequence
  chemically synthesized
MKWVTFISLLFLFSSAYSEVQLLESGGGEVQPGGSLRLSCAASGSVFSIDAMSWFRQAPGKGLELVSAITGGRTTYYAESVKGRFTISRDNAKNTLYLQMSSLRAEDTAVYYCNAVVSTGWGRNADDYWGQGTLVTVKPGGSGGSEVQLLESGGGEVQPGGSLRLSCAASGSVFSIDAMSWFRQAPGKGLELVSAITGGRTTYYAESVKGRFTISRDNAKNTLYLQMSSLRAEDTAVYYCNAVVSTGWGRNADDYWGQGTLVTVKPGGSGGSEVQLLESGGGEVQPGGSLRLSCAASGSVFSIDAMSWFRQAPGKGLELVSAITGGRTTYYAESVKGRFTISRDNAKNTLYLQMSSLRAEDTAVYYCNAVVSTGWGRNADDYWGQGTLVTVKPGGGGDKTHTCPPCPAPGGPSVFLFPPKPKDTLMISRTPEVTCVVVDVSHEDPEVKFNWYVDGVEVHNAKTKPREEQYNSTYRVVSVLTVLHQDWLNGKEYKCKVSNKALPAPIEKTISKAKGQPREPQVYTLPPSRDELTKNQVSLTCLVKGFYPSDIAVEWESNGQPENNYKTTPPVLDSDGSFFLYSKLTVDKSRWQQGNVFSCSVMHEALHNHYTQKSLSLSPGK

SEQ ID NO: 95 - protein, 621 aa, Artificial Sequence
  chemically synthesized
MKWVTFISLLFLFSSAYSEVQLLESGGGEVQPGGSLRLSCAASGSVFSIDAMSWFRQAPGKGLELVCAITGGRTTYYAESVKGRFTCSRDNAKNTLYLQMSSLRAEDTAVYYCNAVVSTGWGRNADDYWGQGTLVTVKPGGSGGSEVQLLESGGGEVQPGGSLRLSCAASGSVFSIDAMSWFRQAPGKGLELVCAITGGRTTYYAESVKGRFTCSRDNAKNTLYLQMSSLRAEDTAVYYCNAVVSTGWGRNADDYWGQGTLVTVKPGGSGGSEVQLLESGGGEVQPGGSLRLSCAASGSVFSIDAMSWFRQAPGKGLELVCAITGGRTTYYAESVKGRFTCSRDNAKNTLYLQMSSLRAEDTAVYYCNAVVSTGWGRNADDYWGQGTLVTVKPGGGGDKTHTCPPCPAPGGPSVFLFPPKPKDTLMISRTPEVTCVVVDVSHEDPEVKFNWYVDGVEVHNAKTKPREEQYNSTYRVVSVLTVLHQDWLNGKEYKCKVSNKALPAPIEKTISKAKGQPREPQVYTLPPSRDELTKNQVSLTCLVKGFYPSDIAVEWESNGQPENNYKTTPPVLDSDGSFFLYSKLTVDKSRWQQGNVFSCSVMHEALHNHYTQKSLSLSPGK

SEQ ID NO: 96 - protein, 624 aa, Artificial Sequence
  chemically synthesized
MKWVTFISLLFLFSSAYSEVQLLESGGGEVQPGGSLRLSCAASGSVFSIDAMSWFRQAPGKGLELVSAITGGRTTYYAESVKGRFTISRDNAKNTLYLQMSSLRAEDTAVYYCNAVVSTGWGRNADDYWGQGTLVTVKPGGSGGSEVQLLESGGGEVQPGGSLRLSCAASGSVFSIDAMSWFRQAPGKGLELVSAITGGRTTYYAESVKGRFTISRDNAKNTLYLQMSSLRAEDTAVYYCNAVVSTGWGRNADDYWGQGTLVTVKPGGSGGSEVQLLESGGGEVQPGGSLRLSCAASGSVFSIDAMSWFRQAPGKGLELVSAITGGRTTYYAESVKGRFTISRDNAKNTLYLQMSSLRAEDTAVYYCNAVVSTGWGRNADDYWGQGTLVTVKPGGGGDKTHTCPPCPAPELLGGPSVFLFPPKPKDTLMISRTPEVTCVVVDVSHEDPEVKFNWYVDGVEVHNAKTKPREEQYNSTYRVVSVLTVLHQDWLNGKEYKCKVSNKALPAPIEKTISKAKGQPREPQVYTLPPSRDELTKNQVSLTCLVKGFYPSDIAVEWESNGQPENNYKTTPPVLDSDGSFFLYSKLTVDKSRWQQGNVFSCSVMHEALHNHYTQKSLSLSPGK

SEQ ID NO: 97 - protein, 624 aa, Artificial Sequence
  chemically synthesized
MKWVTFISLLFLFSSAYSEVQLLESGGGEVQPGGSLRLSCAASGSVFSIDAMSWFRQAPGKGLELVCAITGGRTTYYAESVKGRFTCSRDNAKNTLYLQMSSLRAEDTAVYYCNAVVSTGWGRNADDYWGQGTLVTVKPGGSGGSEVQLLESGGGEVQPGGSLRLSCAASGSVFSIDAMSWFRQAPGKGLELVCAITGGRTTYYAESVKGRFTCSRDNAKNTLYLQMSSLRAEDTAVYYCNAVVSTGWGRNADDYWGQGTLVTVKPGGSGGSEVQLLESGGGEVQPGGSLRLSCAASGSVFSIDAMSWFRQAPGKGLELVCAITGGRTTYYAESVKGRFTCSRDNAKNTLYLQMSSLRAEDTAVYYCNAVVSTGWGRNADDYWGQGTLVTVKPGGGGDKTHTCPPCPAPELLGGPSVFLFPPKPKDTLMISRTPEVTCVVVDVSHEDPEVKFNWYVDGVEVHNAKTKPREEQYNSTYRVVSVLTVLHQDWLNGKEYKCKVSNKALPAPIEKTISKAKGQPREPQVYTLPPSRDELTKNQVSLTCLVKGFYPSDIAVEWESNGQPENNYKTTPPVLDSDGSFFLYSKLTVDKSRWQQGNVFSCSVMHEALHNHYTQKSLSLSPGK

SEQ ID NO: 98 - protein, 621 aa, Artificial Sequence
  chemically synthesized
MKWVTFISLLFLFSSAYSEVQLLESGGGEVQPGGSLRLSCAASGSVFSIDSMSWFRQAPGKGLELVSLITGGRTTYYAESVKGRFTISRDNAKNTLYLQMSSLRAEDTAVYYCNAVVSTGWGRNADDYWGQGTLVTVKPGGSGGSEVQLLESGGGEVQPGGSLRLSCAASGSVFSIDSMSWFRQAPGKGLELVSLITGGRTTYYAESVKGRFTISRDNAKNTLYLQMSSLRAEDTAVYYCNAVVSTGWGRNADDYWGQGTLVTVKPGGSGGSEVQLLESGGGEVQPGGSLRLSCAASGSVFSIDSMSWFRQAPGKGLELVSLITGGRTTYYAESVKGRFTISRDNAKNTLYLQMSSLRAEDTAVYYCNAVVSTGWGRNADDYWGQGTLVTVKPGGGGDKTHTCPPCPAPGGPSVFLFPPKPKDTLMISRTPEVTCVVVDVSHEDPEVKFNWYVDGVEVHNAKTKPREEQYNSTYRVVSVLTVLHQDWLNGKEYKCKVSNKALPAPIEKTISKAKGQPREPQVYTLPPSRDELTKNQVSLTCLVKGFYPSDIAVEWESNGQPENNYKTTPPVLDSDGSFFLYSKLTVDKSRWQQGNVFSCSVMHEALHNHYTQKSLSLSPGK

SEQ ID NO: 99 - protein, 621 aa, Artificial Sequence
  chemically synthesized
MKWVTFISLLFLFSSAYSEVQLLESGGGEVQPGGSLRLSCAASGSVFSIDSMSWFRQAPGKGLELVCLITGGRTTYYAESVKGRFTCSRDNAKNTLYLQMSSLRAEDTAVYYCNAVVSTGWGRNADDYWGQGTLVTVKPGGSGGSEVQLLESGGGEVQPGGSLRLSCAASGSVFSIDSMSWFRQAPGKGLELVCLITGGRTTYYAESVKGRFTCSRDNAKNTLYLQMSSLRAEDTAVYYCNAVVSTGWGRNADDYWGQGTLVTVKPGGSGGSEVQLLESGGGEVQPGGSLRLSCAASGSVFSIDSMSWFRQAPGKGLELVCLITGGRTTYYAESVKGRFTCSRDNAKNTLYLQMSSLRAEDTAVYYCNAVVSTGWGRNADDYWGQGTLVTVKPGGGGDKTHTCPPCPAPGGPSVFLFPPKPKDTLMISRTPEVTCVVVDVSHEDPEVKFNWYVDGVEVHNAKTKPREEQYNSTYRVVSVLTVLHQDWLNGKEYKCKVSNKALPAPIEKTISKAKGQPREPQVYTLPPSRDELTKNQVSLTCLVKGFYPSDIAVEWESNGQPENNYKTTPPVLDSDGSFFLYSKLTVDKSRWQQGNVFSCSVMHEALHNHYTQKSLSLSPGK

SEQ ID NO: 100 - protein, 624 aa, Artificial Sequence
  chemically synthesized
MKWVTFISLLFLFSSAYSEVQLLESGGGEVQPGGSLRLSCAASGSVFSIDSMSWFRQAPGKGLELVSLITGGRTTYYAESVKGRFTISRDNAKNTLYLQMSSLRAEDTAVYYCNAVVSTGWGRNADDYWGQGTLVTVKPGGSGGSEVQLLESGGGEVQPGGSLRLSCAASGSVFSIDSMSWFRQAPGKGLELVSLITGGRTTYYAESVKGRFTISRDNAKNTLYLQMSSLRAEDTAVYYCNAVVSTGWGRNADDYWGQGTLVTVKPGGSGGSEVQLLESGGGEVQPGGSLRLSCAASGSVFSIDSMSWFRQAPGKGLELVSLITGGRTTYYAESVKGRFTISRDNAKNTLYLQMSSLRAEDTAVYYCNAVVSTGWGRNADDYWGQGTLVTVKPGGGGDKTHTCPPCPAPELLGGPSVFLFPPKPKDTLMISRTPEVTCVVVDVSHEDPEVKFNWYVDGVEVHNAKTKPREEQYNSTYRVVSVLTVLHQDWLNGKEYKCKVSNKALPAPIEKTISKAKGQPREPQVYTLPPSRDELTKNQVSLTCLVKGFYPSDIAVEWESNGQPENNYKTTPPVLDSDGSFFLYSKLTVDKSRWQQGNVFSCSVMHEALHNHYTQKSLSLSPGK

SEQ ID NO: 101 - protein, 624 aa, Artificial Sequence
  chemically synthesized
MKWVTFISLLFLFSSAYSEVQLLESGGGEVQPGGSLRLSCAASGSVFSIDSMSWFRQAPGKGLELVCLITGGRTTYYAESVKGRFTCSRDNAKNTLYLQMSSLRAEDTAVYYCNAVVSTGWGRNADDYWGQGTLVTVKPGGSGGSEVQLLESGGGEVQPGGSLRLSCAASGSVFSIDSMSWFRQAPGKGLELVCLITGGRTTYYAESVKGRFTCSRDNAKNTLYLQMSSLRAEDTAVYYCNAVVSTGWGRNADDYWGQGTLVTVKPGGSGGSEVQLLESGGGEVQPGGSLRLSCAASGSVFSIDSMSWFRQAPGKGLELVCLITGGRTTYYAESVKGRFTCSRDNAKNTLYLQMSSLRAEDTAVYYCNAVVSTGWGRNADDYWGQGTLVTVKPGGGGDKTHTCPPCPAPELLGGPSVFLFPPKPKDTLMISRTPEVTCVVVDVSHEDPEVKFNWYVDGVEVHNAKTKPREEQYNSTYRVVSVLTVLHQDWLNGKEYKCKVSNKALPAPIEKTISKAKGQPREPQVYTLPPSRDELTKNQVSLTCLVKGFYPSDIAVEWESNGQPENNYKTTPPVLDSDGSFFLYSKLTVDKSRWQQGNVFSCSVMHEALHNHYTQKSLSLSPGK

SEQ ID NO: 102 - protein, 621 aa, Artificial Sequence
  chemically synthesized
MKWVTFISLLFLFSSAYSEVQLLESGGGEVQPGGSLRLSCAASGSVFSIDAMSWFRQAPGKGLELVSLITGGRTTYYAESVKGRFTISRDNAKNTLYLQMSSLRAEDTAVYYCNAVVSTGWGRNADDYWGQGTLVTVKPGGSGGSEVQLLESGGGEVQPGGSLRLSCAASGSVFSIDAMSWFRQAPGKGLELVSLITGGRTTYYAESVKGRFTISRDNAKNTLYLQMSSLRAEDTAVYYCNAVVSTGWGRNADDYWGQGTLVTVKPGGSGGSEVQLLESGGGEVQPGGSLRLSCAASGSVFSIDAMSWFRQAPGKGLELVSLITGGRTTYYAESVKGRFTISRDNAKNTLYLQMSSLRAEDTAVYYCNAVVSTGWGRNADDYWGQGTLVTVKPGGGGDKTHTCPPCPAPGGPSVFLFPPKPKDTLMISRTPEVTCVVVDVSHEDPEVKFNWYVDGVEVHNAKTKPREEQYNSTYRVVSVLTVLHQDWLNGKEYKCKVSNKALPAPIEKTISKAKGQPREPQVYTLPPSRDELTKNQVSLTCLVKGFYPSDIAVEWESNGQPENNYKTTPPVLDSDGSFFLYSKLTVDKSRWQQGNVFSCSVMHEALHNHYTQKSLSLSPGK

SEQ ID NO: 103 - protein, 621 aa, Artificial Sequence
  chemically synthesized
MKWVTFISLLFLFSSAYSEVQLLESGGGEVQPGGSLRLSCAASGSVFSIDAMSWFRQAPGKGLELVCLITGGRTTYYAESVKGRFTCSRDNAKNTLYLQMSSLRAEDTAVYYCNAVVSTGWGRNADDYWGQGTLVTVKPGGSGGSEVQLLESGGGEVQPGGSLRLSCAASGSVFSIDAMSWFRQAPGKGLELVCLITGGRTTYYAESVKGRFTCSRDNAKNTLYLQMSSLRAEDTAVYYCNAVVSTGWGRNADDYWGQGTLVTVKPGGSGGSEVQLLESGGGEVQPGGSLRLSCAASGSVFSIDAMSWFRQAPGKGLELVCLITGGRTTYYAESVKGRFTCSRDNAKNTLYLQMSSLRAEDTAVYYCNAVVSTGWGRNADDYWGQGTLVTVKPGGGGDKTHTCPPCPAPGGPSVFLFPPKPKDTLMISRTPEVTCVVVDVSHEDPEVKFNWYVDGVEVHNAKTKPREEQYNSTYRVVSVLTVLHQDWLNGKEYKCKVSNKALPAPIEKTISKAKGQPREPQVYTLPPSRDELTKNQVSLTCLVKGFYPSDIAVEWESNGQPENNYKTTPPVLDSDGSFFLYSKLTVDKSRWQQGNVFSCSVMHEALHNHYTQKSLSLSPGK

SEQ ID NO: 104 - protein, 624 aa, Artificial Sequence
  chemically synthesized
MKWVTFISLLFLFSSAYSEVQLLESGGGEVQPGGSLRLSCAASGSVFSIDAMSWFRQAPGKGLELVSLITGGRTTYYAESVKGRFTISRDNAKNTLYLQMSSLRAEDTAVYYCNAVVSTGWGRNADDYWGQGTLVTVKPGGSGGSEVQLLESGGGEVQPGGSLRLSCAASGSVFSIDAMSWFRQAPGKGLELVSLITGGRTTYYAESVKGRFTISRDNAKNTLYLQMSSLRAEDTAVYYCNAVVSTGWGRNADDYWGQGTLVTVKPGGSGGSEVQLLESGGGEVQPGGSLRLSCAASGSVFSIDAMSWFRQAPGKGLELVSLITGGRTTYYAESVKGRFTISRDNAKNTLYLQMSSLRAEDTAVYYCNAVVSTGWGRNADDYWGQGTLVTVKPGGGGDKTHTCPPCPAPELLGGPSVFLFPPKPKDTLMISRTPEVTCVVVDVSHEDPEVKFNWYVDGVEVHNAKTKPREEQYNSTYRVVSVLTVLHQDWLNGKEYKCKVSNKALPAPIEKTISKAKGQPREPQVYTLPPSRDELTKNQVSLTCLVKGFYPSDIAVEWESNGQPENNYKTTPPVLDSDGSFFLYSKLTVDKSRWQQGNVFSCSVMHEALHNHYTQKSLSLSPGK

SEQ ID NO: 105 - protein, 624 aa, Artificial Sequence
  chemically synthesized
MKWVTFISLLFLFSSAYSEVQLLESGGGEVQPGGSLRLSCAASGSVFSIDAMSWFRQAPGKGLELVCLITGGRTTYYAESVKGRFTCSRDNAKNTLYLQMSSLRAEDTAVYYCNAVVSTGWGRNADDYWGQGTLVTVKPGGSGGSEVQLLESGGGEVQPGGSLRLSCAASGSVFSIDAMSWFRQAPGKGLELVCLITGGRTTYYAESVKGRFTCSRDNAKNTLYLQMSSLRAEDTAVYYCNAVVSTGWGRNADDYWGQGTLVTVKPGGSGGSEVQLLESGGGEVQPGGSLRLSCAASGSVFSIDAMSWFRQAPGKGLELVCLITGGRTTYYAESVKGRFTCSRDNAKNTLYLQMSSLRAEDTAVYYCNAVVSTGWGRNADDYWGQGTLVTVKPGGGGDKTHTCPPCPAPELLGGPSVFLFPPKPKDTLMISRTPEVTCVVVDVSHEDPEVKFNWYVDGVEVHNAKTKPREEQYNSTYRVVSVLTVLHQDWLNGKEYKCKVSNKALPAPIEKTISKAKGQPREPQVYTLPPSRDELTKNQVSLTCLVKGFYPSDIAVEWESNGQPENNYKTTPPVLDSDGSFFLYSKLTVDKSRWQQGNVFSCSVMHEALHNHYTQKSLSLSPGK

SEQ ID NO: 106 - protein, 9 aa, Artificial Sequence
  chemically synthesized
GSVFSIDAM

SEQ ID NO: 107 - protein, 8 aa, Artificial Sequence
  chemically synthesized
VMSSGSPK

SEQ ID NO: 108 - protein, 16 aa, Artificial Sequence
  chemically synthesized
YADVATGWGRDASAYW

SEQ ID NO: 109 - protein, 10 aa, Artificial Sequence
  chemically synthesized
AGSTFSVNSM

SEQ ID NO: 110 - protein, 8 aa, Artificial Sequence
  chemically synthesized
FTGGSTMN

SEQ ID NO: 111 - protein, 16 aa, Artificial Sequence
  chemically synthesized
NAEVNEGWNADYHDYW

SEQ ID NO: 112 - protein, 10 aa, Artificial Sequence
  chemically synthesized
SGSIFSINHM

SEQ ID NO: 113 - protein, 9 aa, Artificial Sequence
  chemically synthesized
HITGGASTK

SEQ ID NO: 114 - protein, 16 aa, Artificial Sequence
  chemically synthesized
NAEVNEGWNADYYDVW

SEQ ID NO: 115 - protein, 9 aa, Artificial Sequence
  chemically synthesized
VLNGISSAK

SEQ ID NO: 116 - protein, 16 aa, Artificial Sequence
  chemically synthesized
YADVSTGWGRDAHGYW

SEQ ID NO: 117 - protein, 10 aa, Artificial Sequence
  chemically synthesized
SGNIFSIDAM

SEQ ID NO: 118 - protein, 5 aa, Artificial Sequence
  chemically synthesized
QIPGG

SEQ ID NO: 119 - protein, 16 aa, Artificial Sequence
  chemically synthesized
NIVASTSWGSPSKVYW

SEQ ID NO: 120 - protein, 10 aa, Artificial Sequence
  chemically synthesized
SGSVFSIDSM

SEQ ID NO: 121 - protein, 9 aa, Artificial Sequence
  chemically synthesized
LITGGRTTT

SEQ ID NO: 122 - protein, 16 aa, Artificial Sequence
  chemically synthesized
NAVVSTGWGRNADDYW

SEQ ID NO: 123 - protein, 8 aa, Artificial Sequence
  chemically synthesized
VIDGVSPN

SEQ ID NO: 124 - protein, 16 aa, Artificial Sequence
  chemically synthesized
NAAVSTGWGRNADDYW

SEQ ID NO: 125 - protein, 10 aa, Artificial Sequence
  chemically synthesized
SGSVFSIDSV

SEQ ID NO: 126 - protein, 16 aa, Artificial Sequence
  chemically synthesized
NAALSTGWGRDASAYW

SEQ ID NO: 127 - protein, 15 aa, Artificial Sequence
  chemically synthesized
AEVNEGWNADYYDVW

SEQ ID NO: 128 - protein, 8 aa, Artificial Sequence
  chemically synthesized
ITSGGSPN

SEQ ID NO: 129 - protein, 15 aa, Artificial Sequence
  chemically synthesized
AGELRDDSNGYLHYW

SEQ ID NO: 130 - protein, 9 aa, Artificial Sequence
  chemically synthesized
HITGGRTTT

SEQ ID NO: 131 - protein, 10 aa, Artificial Sequence
  chemically synthesized
SGSIFSIDDM

SEQ ID NO: 132 - protein, 8 aa, Artificial Sequence
  chemically synthesized
VHSGSSTN

SEQ ID NO: 133 - protein, 16 aa, Artificial Sequence
  chemically synthesized
YAAISSGWGRDAEDYW

SEQ ID NO: 134 - protein, 8 aa, Artificial Sequence
  chemically synthesized
ITGGRTTT

SEQ ID NO: 135 - protein, 16 aa, Artificial Sequence
  chemically synthesized
NAAVSTGWGRSADDYW

SEQ ID NO: 136 - protein, 8 aa, Artificial Sequence
  chemically synthesized
ITGGRTTY

SEQ ID NO: 137 - protein, 9 aa, Artificial Sequence
  chemically synthesized
AITGGRTTY

SEQ ID NO: 138 - protein, 10 aa, Artificial Sequence
  chemically synthesized
SGSVFSIDAM

SEQ ID NO: 139 - protein, 8 aa, Artificial Sequence
  chemically synthesized
LSGISSAT

SEQ ID NO: 140 - protein, 15 aa, Artificial Sequence
  chemically synthesized
ADVSTGWGRDAHGYW

SEQ ID NO: 141 - protein, 8 aa, Artificial Sequence
  chemically synthesized
LSGISSAK

SEQ ID NO: 142 - protein, 15 aa, Artificial Sequence
  chemically synthesized
ADVSTGWGRDAHGYW

SEQ ID NO: 143 - protein, 10 aa, Artificial Sequence
  chemically synthesized
SGFTFSTHGM

SEQ ID NO: 144 - protein, 10 aa, Artificial Sequence
  chemically synthesized
AINNGGSWTS

SEQ ID NO: 145 - protein, 7 aa, Artificial Sequence
  chemically synthesized
CQNRVTR

SEQ ID NO: 146 - protein, 6 aa, Artificial Sequence
  chemically synthesized
QNRVTR

SEQ ID NO: 147 - protein, 9 aa, Artificial Sequence
  chemically synthesized
INQGGSWTS

SEQ ID NO: 148 - protein, 10 aa, Artificial Sequence
  chemically synthesized
SRSIASINVM

SEQ ID NO: 149 - protein, 10 aa, Artificial Sequence
  chemically synthesized
SGSIFSIDAM

SEQ ID NO: 150 - protein, 16 aa, Artificial Sequence
  chemically synthesized
NADVSTGWGRPADHYW